European Patent Application EP 4 209 581 A1, published July 12, 2023. Title: MICROBIAL CONSORTIA PRODUCING DIPICOLINIC ACID AND METHODS FOR SELECTING MICROBES FOR CO-FORMULATION WITH CARRIERS. Applicant: AMVAC Hong Kong Limited. Application EP. The sequence listing filed with the application follows.

SEQUENCE LISTING (67 sequences)

SEQ ID NO: 1 - DNA, 1524 bp, Streptomyces pratensis
  source 1..1524: mol_type = unassigned DNA
catggagagtttgatcctggctcaggacgaacgctggcggcgtgcttaacacatgcaagtcgaacgatgaagcccttcggggtggattagtggcgaacgggtgagtaacacgtgggcaatctgcccttcactctgggacaagccctggaaacggggtctaataccggataacactctgtccctcatggggcggggttaaaagctccggcggtgaaggatgagcccgcggcctatcagcttgttggtggggtaatggcctaccaaggcgacgacgggtagccggcctgagagggcgaccggccacactgggactgagacacggcccagactcctacgggaggcagcagtggggaatattgcacaatgggcgaaagcctgatgcagcgacgccgcgtgagggatgacggccttcgggttgtaaacctctttcagcagggaagaagcgcaagtgacggtacctgcagaagaagcaccggctaactacgtgccagcagccgcggtaatacgtagggtgcgagcgttgtccggaattattgggcgtaaagagctcgtaggcggcttgtcacgtcggatgtgaaagctcggggcttaaccccgagtctgcattcgatacgggctagctagagtgtggtaggggagatcggaattcctggtgtagcggtgaaatgcgcagatatcaggaggaacaccggtggcgaaggcggatctctgggccattactgacgctgaggagcgaaagcgtggggagcgaacaggattagataccctggtagtccacgccgtaaacgttgggaactaggtgttggcgacattccacgtcgtcggtgccgcagctaacgcattaagttccccgcctggggagtacggccgcaaggctaaaactcaaaggaattgacgggggcccgcacaagcagcggagcatgtggcttaattcgacgcaacgcgaagaaccttaccaaggcttgacatataccggaaagcatcagagatggtgccccccttgtggtcggtatacaggtggtgcatggctgtcgtcagctcgtgtcgtgagatgttgggttaagtcccgcaacgagcgcaacccttgttctgtgttgccagcatgcccttcggggtgatggggactcacaggagactgccggggtcaactcggaggaaggtggggacgacgtcaagtcatcatgccccttatgtcttgggctgcacacgtgctacaatggccggtacaatgagctgcgatgccgcgaggcggagcgaatctcaaaaagccggtctcagttcggattggggtctgcaactcgaccccatgaagtcggagttgctagtaatcgcagatcagcattgctgcggtgaatacgttcccgggccttgtacacaccgcccgtcacgtcacgaaagtcggtaacacccgaagccggtggcccaaccccttgtgggagggagctgtcgaaggtgggactggcgattgggacgaagtcgtaacaaggtagccgtaccggaaggtgcggctggatcacctccttt

SEQ ID NO: 2 - DNA, 1524 bp, Streptomyces venezuelae
  source 1..1524: mol_type = unassigned DNA
cacggagagtttgatcctggctcaggacgaacgctggcggcgtgcttaacacatgcaagtcgaacgatgaagcccttcggggtggattagtggcgaacgggtgagtaacacgtgggcaatctgcccttcactctgggacaagccctggaaacggggtctaataccggataacaccggctcctgcatgggggctggttaaaagctccggcggtgaaggatgagcccgcggcctatcagcttgttggtggggtaatggcctaccaaggcgacgacgggtagccggcctgagagggcgaccggccacactgggactgagacacggcccagactcctacgggaggcagcagtggggaatattgcacaatgggcgaaagcctgatgcagcgacgccgcgtgagggatgacggccttcgggttgtaaacctctttcagcagggaagaagcgaaagtgacggtacctgcagaagaagcgccggctaactacgtgccagcagccgcggtaatacgtagggcgcaagcgttgtccggaattattgggcgtaaagagctcgtaggcggcttgtcacgtcgggtgtgaaagcccggggcttaaccccgggtctgcatccgatacgggcaggctagagtgtggtaggggagatcggaattcctggtgtagcggtgaaatgcgcagatatcaggaggaacaccggtggcgaaggcggatctctgggccattactgacgctgaggagcgaaagcgtggggagcgaacaggattagataccctggtagtccacgccgtaaacgttgggaactaggtgttggcgacattccacgtcgtcggtgccgcagctaacgcattaagttccccgcctggggagtacggccgcaaggctaaaactcaaaggaattgacgggggcccgcacaagcagcggagcatgtggcttaattcgacgcaacgcgaagaaccttaccaaggcttgacatataccggaaagcattagagatagtgccccccttgtggtcggtatacaggtggtgcatggctgtcgtcagctcgtgtcgtgagatgttgggttaagtcccgcaacgagcgcaacccttgtcctgtgttgccagcatgcccttcggggtgatggggactcacaggagaccgccggggtcaactcggaggaaggtggggacgacgtcaagtcatcatgccccttatgtcttgggctgcacacgtgctacaatggccggtacaaagagctgcgatgccgtgaggcggagcgaatctcaaaaagccggtctcagttcggattggggtctgcaactcgaccccatgaagtcggagttgctagtaatcgcagatcagcattgctgcggtgaatacgttcccgggccttgtacacaccgcccgtcacgtcacgaaagtcggtaacacccgaagccggtggcccaaccccttgtgggagggagctgtcgaaggtgggactggcgattgggacgaagtcgtaacaaggtagccgtaccggaaggtgcggctggatcacctccttt

SEQ ID NO: 3 - DNA, 1548 bp, Bacillus firmus
  source 1..1548: mol_type = unassigned DNA
tatggagagtttgatcctggctcaggacgaacgctggcggcgtgcctaatacatgcaagtcgagcggacagatgggagcttgctccctgaagtcagcggcggacgggtgagtaacacgtgggcaacctgcctgtaagactgggataactccgggaaaccggggctaataccggataattctttccctcacatgagggaaagctgaaagatggtttcggctatcacttacagatgggcccgcggcgcattagctagttggtgaggtaacggctcaccaaggcaacgatgcgtagccgacctgagagggtgatcggccacactgggactgagacacggcccagactcctacgggaggcagcagtagggaatcttccgcaatggacgaaagtctgacggagcaacgccgcgtgagtgatgaaggttttcggatcgtaaaactctgttgttagggaagaacaagtaccggagtaactgccggtaccttgacggtacctaaccagaaagccacggctaactacgtgccagcagccgcggtaatacgtaggtggcaagcgttgtccggaattattgggcgtaaagcgcgcgcaggcggttccttaagtctgatgtgaaagcccccggctcaaccggggagggtcattggaaactggggaacttgagtgcagaagagaagagtggaattccacgtgtagcggtgaaatgcgtagagatgtggaggaacaccagtggcgaaggcgactctttggtctgtaactgacgctgaggcgcgaaagcgtggggagcaaacaggattagataccctggtagtccacgccgtaaacgatgagtgctaagtgttagagggtttccgccctttagtgctgcagcaaacgcattaagcactccgcctggggagtacggccgcaaggctgaaactcaaaggaattgacgggggcccgcacaagcggtggagcatgtggtttaattcgaagcaacgcgaagaaccttaccaggtcttgacatctcctgacaaccctagagatagggcgttccccttcgggggacaggatgacaggtggtgcatggttgtcgtcagctcgtgtcgtgagatgttgggttaagtcccgcaacgagcgcaacccttgatcttagttgccagcattcagttgggcactctaaggtgactgccggtgacaaaccggaggaaggtggggatgacgtcaaatcatcatgccccttatgacctgggctacacacgtgctacaatggatggtacaaagggctgcgagaccgcgaggttaagcgaatcccataaaaccattctcagttcggattgcaggctgcaactcgcctgcatgaagccggaatcgctagtaatcgcggatcagcatgccgcggtgaatacgttcccgggccttgtacacaccgcccgtcacaccacgagagtttgtaacacccgaagtcggtggggtaaccttttggagccagccgcctaaggtgggacagatgattggggtgaagtcgtaacaaggtagccgtatcggaaggtgcggctggatcacctccttt

SEQ ID NO: 4 - DNA, 1552 bp, Paenibacillus azoreducens
  source 1..1552: mol_type = unassigned DNA
cttggagagtttgatcctggctcaggacgaacgctggcggcgtgcctaatacatgcaagtcgagcggatttgatgaggagcttgctcctctgatggttagcggcggacgggtgagtaacacgtaggcaacctgcctgcaagaccgggataactagcggaaacgttagctaataccggataatttatcgctttgcatgaagcgataatgaaagacggagcaatctgtcacttgcagatgggcctgcggcgcattagctagttggtgaggtaacggctcaccaaggcgacgatgcgtagccgacctgagagggtgaacggccacactgggactgagacacggcccagactcctacgggaggcagcagtagggaatcttccgcaatgggcgaaagcctgacggagcaacgccgcgtgagtgatgaaggttttcggatcgtaaagctctgttgccagggaagaacgaccgttagagtaactgctaacggagtgacggtacctgagaagaaagccccggctaactacgtgccagcagccgcggtaatacgtagggggcaagcgttgtccggaattattgggcgtaaagcgcgcgcaggcggtcgcttaagtctggtgtttaaggccaaggctcaaccttggttcgcactggaaactgggtgacttgagtgcagaagaggagagtggaattccacgtgtagcggtgaaatgcgtagagatgtggaggaacaccagtggcgaaggcgactctctgggctgtaactgacgctgaggcgcgaaagcgtggggagcaaacaggattagataccctggtagtccacgccgtaaacgatgaatgctaggtgttaggggtttcgatacccttggtgccgaagttaacacattaagcattccgcctggggagtacggtcgcaagactgaaactcaaaggaattgacggggacccgcacaagcagtggagtatgtggtttaattcgaagcaacgcgaagaaccttaccaggtcttgacatccctctgaccggactagagatagtcctttccttcgggacagaggagacaggtggtgcatggttgtcgtcagctcgtgtcgtgagatgttgggttaagtcccgcaacgagcgcaacccttgattttagttgccagcactttaaggtgggcactctaaaatgactgccggtgacaaaccggaggaaggcggggatgacgtcaaatcatcatgccccttatgacctgggctacacacgtactacaatggccagtacaacgggaagcgaaatcgcgagatggagccaatcctatcaaagctggtctcagttcggattgcaggctgcaactcgcctgcatgaagtcggaattgctagtaatcgcggatcagcatgccgcggtgaatacgttcccgggtcttgtacacaccgcccgtcacaccacgagagtttacaacacccgaagtcggtgaggtaaccgcaaggagccagccgccgaaggtggggtagatgattggggtgaagtcgtaacaaggtagccgtatcggaaggtgcggctggatcacctccttt

SEQ ID NO: 5 - DNA, 1548 bp, Bacillus amyloliquefaciens
  source 1..1548: mol_type = unassigned DNA
atcggagagtttgatcctggctcaggacgaacgctggcggcgtgcctaatacatgcaagtcgagcggacagatgggagcttgctccctgatgttagcggcggacgggtgagtaacacgtgggtaacctgcctgtaagactgggataactccgggaaaccggggctaataccggatggttgtctgaaccgcatggttcagacataaaaggtggcttcggctaccacttacagatggacccgcggcgcattagctagttggtgaggtaacggctcaccaaggcgacgatgcgtagccgacctgagagggtgatcggccacactgggactgagacacggcccagactcctacgggaggcagcagtagggaatcttccgcaatggacgaaagtctgacggagcaacgccgcgtgagtgatgaaggttttcggatcgtaaagctctgttgttagggaagaacaagtgccgttcaaatagggcggcaccttgacggtacctaaccagaaagccacggctaactacgtgccagcagccgcggtaatacgtaggtggcaagcgttgtccggaattattgggcgtaaagggctcgcaggcggtttcttaagtctgatgtgaaagcccccggctcaaccggggagggtcattggaaactggggaacttgagtgcagaagaggagagtggaattccacgtgtagcggtgaaatgcgtagagatgtggaggaacaccagtggcgaaggcgactctctggtctgtaactgacgctgaggagcgaaagcgtggggagcgaacaggattagataccctggtagtccacgccgtaaacgatgagtgctaagtgttagggggtttccgccccttagtgctgcagctaacgcattaagcactccgcctggggagtacggtcgcaagactgaaactcaaaggaattgacgggggcccgcacaagcggtggagcatgtggtttaattcgaagcaacgcgaagaaccttaccaggtcttgacatcctctgacaatcctagagataggacgtccccttcgggggcagagtgacaggtggtgcatggttgtcgtcagctcgtgtcgtgagatgttgggttaagtcccgcaacgagcgcaacccttgatcttagttgccagcattcagttgggcactctaaggtgactgccggtgacaaaccggaggaaggtggggatgacgtcaaatcatcatgccccttatgacctgggctacacacgtgctacaatggacagaacaaagggcagcgaaaccgcgaggttaagccaatcccacaaatctgttctcagttcggatcgcagtctgcaactcgactgcgtgaagctggaatcgctagtaatcgcggatcagcatgccgcggtgaatacgttcccgggccttgtacacaccgcccgtcacaccacgagagtttgtaacacccgaagtcggtgaggtaacctttatggagccagccgccgaaggtgggacagatgattggggtgaagtcgtaacaaggtagccgtatcggaaggtgcggctggatcacctccttt

SEQ ID NO: 6 - DNA, 1550 bp, Bacillus flexus
  source 1..1550: mol_type = unassigned DNA
tcggagagtttgatcctggctcaggatgaacgctggcggcgtgcctaatacatgcaagtcgagcgaactgattagaagcttgcttctatgacgttagcggcggacgggtgagtaacacgtgggcaacctgcctgtaagactgggataactccgggaaaccggagctaataccggataacattttctcttgcataagagaaaattgaaagatggtttcggctatcacttacagatgggcccgcggtgcattagctagttggtgaggtaacggctcaccaaggcaacgatgcatagccgacctgagagggtgatcggccacactgggactgagacacggcccagactcctacgggaggcagcagtagggaatcttccgcaatggacgaaagtctgacggagcaacgccgcgtgagtgatgaaggctttcgggtcgtaaaactctgttgttagggaagaacaagtacaagagtaactgcttgtaccttgacggtacctaaccagaaagccacggctaactacgtgccagcagccgcggtaatacgtaggtggcaagcgttatccggaattattgggcgtaaagcgcgcgcaggcggtttcttaagtctgatgtgaaagcccacggctcaaccgtggagggtcattggaaactggggaacttgagtgcagaagagaaaagcggaattccacgtgtagcggtgaaatgcgtagagatgtggaggaacaccagtggcgaaggcggctttttggtctgtaactgacgctgaggcgcgaaagcgtggggagcaaacaggattagataccctggtagtccacgccgtaaacgatgagtgctaagtgttagagggtttccgccctttagtgctgcagctaacgcattaagcactccgcctggggagtacggtcgcaagactgaaactcaaaggaattgacgggggcccgcacaagcggtggagcatgtggtttaattcgaagcaacgcgaagaaccttaccaggtcttgacatcctctgacaactctagagatagagcgttccccttcgggggacagagtgacaggtggtgcatggttgtcgtcagctcgtgtcgtgagatgttgggttaagtcccgcaacgagcgcaacccttgatcttagttgccagcatttagttgggcactctaaggtgactgccggtgacaaaccggaggaaggtggggatgacgtcaaatcatcatgccccttatgacctgggctacacacgtgctacaatggatggtacaaagggctgcaagaccgcgaggtcaagccaatcccataaaaccattctcagttcggattgtaggctgcaactcgcctacatgaagctggaatcgctagtaatcgcggatcagcatgccgcggtgaatacgttcccgggccttgtacacaccgcccgtcacaccacgagagtttgtaacacccgaagtcggtggggtaacctttatggagccagccgcctaaggtgggacagatgattggggtgaagtcgtaacaaggtagccgtatcggaaggtgcggctggatcacctccttt

SEQ ID NO: 7 - DNA, 1549 bp, Bacillus licheniformis
  source 1..1549: mol_type = unassigned DNA
catggagagtttgatcctggctcaggacgaacgctggcggcgtgcctaatacatgcaagtcgagcggaccgacgggagcttgctcccttaggtcagcggcggacgggtgagtaacacgtgggtaacctgcctgtaagactgggataactccgggaaaccggggctaataccggatgcttgattgaaccgcatggttccaatcataaaaggtggcttttagctaccacttacagatggacccgcggcgcattagctagttggtgaggtaacggctcaccaaggcgacgatgcgtagccgacctgagagggtgatcggccacactgggactgagacacggcccagactcctacgggaggcagcagtagggaatcttccgcaatggacgaaagtctgacggagcaacgccgcgtgagtgatgaaggttttcggatcgtaaaactctgttgttagggaagaacaagtaccgttcgaatagggcggcaccttgacggtacctaaccagaaagccacggctaactacgtgccagcagccgcggtaatacgtaggtggcaagcgttgtccggaattattgggcgtaaagcgcgcgcaggcggtttcttaagtctgatgtgaaagcccccggctcaaccggggagggtcattggaaactggggaacttgagtgcagaagaggagagtggaattccacgtgtagcggtgaaatgcgtagagatgtggaggaacaccagtggcgaaggcgactctctggtctgtaactgacgctgaggcgcgaaagcgtggggagcgaacaggattagataccctggtagtccacgccgtaaacgatgagtgctaagtgttagagggtttccgccctttagtgctgcagcaaacgcattaagcactccgcctggggagtacggtcgcaagactgaaactcaaaggaattgacgggggcccgcacaagcggtggagcatgtggtttaattcgaagcaacgcgaagaaccttaccaggtcttgacatcctctgacaaccctagagatagggcttccccttcgggggcagagtgacaggtggtgcatggttgtcgtcagctcgtgtcgtgagatgttgggttaagtcccgcaacgagcgcaacccttgatcttagttgccagcattcagttgggcactctaaggtgactgccggtgacaaaccggaggaaggtggggatgacgtcaaatcatcatgccccttatgacctgggctacacacgtgctacaatgggcagaacaaagggcagcgaagccgcgaggctaagccaatcccacaaatctgttctcagttcggatcgcagtctgcaactcgactgcgtgaagctggaatcgctagtaatcgcggatcagcatgccgcggtgaatacgttcccgggccttgtacacaccgcccgtcacaccacgagagtttgtaacacccgaagtcggtgaggtaaccttttggagccagccgccgaaggtgggacagatgattggggtgaagtcgtaacaaggtagccgtatcggaaggtgcggctggatcacctccttt

SEQ ID NO: 8 - DNA, 1549 bp, Bacillus megaterium
  source 1..1549: mol_type = unassigned DNA
tcggagagtttgatcctggctcaggatgaacgctggcggcgtgcctaatacatgcaagtcgagcgaactgattagaagcttgcttctatgacgttagcggcggacgggtgagtaacacgtgggcaacctgcctgtaagactgggataacttcgggaaaccgaagctaataccggataggatcttctccttcatgggagatgattgaaagatggtttcggctatcacttacagatgggcccgcggtgcattagctagttggtgaggtaacggctcaccaaggcaacgatgcatagccgacctgagagggtgatcggccacactgggactgagacacggcccagactcctacgggaggcagcagtagggaatcttccgcaatggacgaaagtctgacggagcaacgccgcgtgagtgatgaaggctttcgggtcgtaaaactctgttgttagggaagaacaagtacgagagtaactgctcgtaccttgacggtacctaaccagaaagccacggctaactacgtgccagcagccgcggtaatacgtaggtggcaagcgttatccggaattattgggcgtaaagcgcgcgcaggcggtttcttaagtctgatgtgaaagcccacggctcaaccgtggagggtcattggaaactggggaacttgagtgcagaagagaaaagcggaattccacgtgtagcggtgaaatgcgtagagatgtggaggaacaccagtggcgaaggcggctttttggtctgtaactgacgctgaggcgcgaaagcgtggggagcaaacaggattagataccctggtagtccacgccgtaaacgatgagtgctaagtgttagagggtttccgccctttagtgctgcagctaacgcattaagcactccgcctggggagtacggtcgcaagactgaaactcaaaggaattgacgggggcccgcacaagcggtggagcatgtggtttaattcgaagcaacgcgaagaaccttaccaggtcttgacatcctctgacaactctagagatagagcgttccccttcgggggacagagtgacaggtggtgcatggttgtcgtcagctcgtgtcgtgagatgttgggttaagtcccgcaacgagcgcaacccttgatcttagttgccagcatttagttgggcactctaaggtgactgccggtgacaaaccggaggaaggtggggatgacgtcaaatcatcatgccccttatgacctgggctacacacgtgctacaatggatggtacaaagggctgcaagaccgcgaggtcaagccaatcccataaaaccattctcagttcggattgtaggctgcaactcgcctacatgaagctggaatcgctagtaatcgcggatcagcatgccgcggtgaatacgttcccgggccttgtacacaccgcccgtcacaccacgagagtttgtaacacccgaagtcggtggagtaaccgtaaggagctagccgcctaaggtgggacagatgattggggtgaagtcgtaacaaggtagccgtatcggaaggtgcggctggatcacctccttt

SEQ ID NO: 9 - DNA, 1544 bp, Bacillus pumilus
  source 1..1544: mol_type = unassigned DNA
ggagagtttgatcctggctcaggacgaacgctggcggcgtgcctaatacatgcaagtcgagcggacagaagggagcttgctcccggatgttagcggcggacgggtgagtaacacgtgggtaacctgcctgtaagactgggataactccgggaaaccggagctaataccggatagttccttgaaccgcatggttcaaggatgaaagacggtttcggctgtcacttacagatggacccgcggcgcattagctagttggtggggtaatggctcaccaaggcgacgatgcgtagccgacctgagagggtgatcggccacactgggactgagacacggcccagactcctacgggaggcagcagtagggaatcttccgcaatggacgaaagtctgacggagcaacgccgcgtgagtgatgaaggttttcggatcgtaaagctctgttgttagggaagaacaagtgcgagagtaactgctcgcaccttgacggtacctaaccagaaagccacggctaactacgtgccagcagccgcggtaatacgtaggtggcaagcgttgtccggaattattgggcgtaaagggctcgcaggcggtttcttaagtctgatgtgaaagcccccggctcaaccggggagggtcattggaaactgggaaacttgagtgcagaagaggagagtggaattccacgtgtagcggtgaaatgcgtagagatgtggaggaacaccagtggcgaaggcgactctctggtctgtaactgacgctgaggagcgaaagcgtggggagcgaacaggattagataccctggtagtccacgccgtaaacgatgagtgctaagtgttagggggtttccgccccttagtgctgcagctaacgcattaagcactccgcctggggagtacggtcgcaagactgaaactcaaaggaattgacgggggcccgcacaagcggtggagcatgtggtttaattcgaagcaacgcgaagaaccttaccaggtcttgacatcctctgacaaccctagagatagggctttcccttcggggacagagtgacaggtggtgcatggttgtcgtcagctcgtgtcgtgagatgttgggttaagtcccgcaacgagcgcaacccttgatcttagttgccagcatttagttgggcactctaaggtgactgccggtgacaaaccggaggaaggtggggatgacgtcaaatcatcatgccccttatgacctgggctacacacgtgctacaatggacagaacaaagggctgcgagaccgcaaggtttagccaatcccataaatctgttctcagttcggatcgcagtctgcaactcgactgcgtgaagctggaatcgctagtaatcgcggatcagcatgccgcggtgaatacgttcccgggccttgtacacaccgcccgtcacaccacgagagtttgcaacacccgaagtcggtgaggtaacctttatggagccagccgccgaaggtggggcagatgattggggtgaagtcgtaacaaggtagccgtatcggaaggtgcggctggatcacctccttt

SEQ ID NO: 10 - DNA, 1549 bp, Bacillus koreensis
  source 1..1549: mol_type = unassigned DNA
tcggagagtttgatcctggctcaggacgaacgctggcggcgtgcctaatacatgcaagtcgagcggacttgttagaagcttgcttctaacaagttagcggcggacgggtgagtaacacgtgggtaacctgcctgtaagatggggataactccgggaaaccggagctaataccgaataacactttcgctcgcatgagcggatgttaaaagacggtttcggctgtcacttacagatggacccgcggcgcattagctagttggtgaggtaacggctcaccaaggcgacgatgcgtagccgacctgagagggtgatcggccacactgggactgagacacggcccagactcctacgggaggcagcagtagggaatcttccgcaatggacgaaagtctgacggagcaacgccgcgtgagtgatgaaggttttcggatcgtaaaactctgttgttagggaagaacaagtacgagagtaactgctcgtaccttgacggtacctaaccagaaagccacggctaactacgtgccagcagccgcggtaatacgtaggtggcaagcgttgtccggaattattgggcgtaaagcgcgcgcaggcggttccttaagtctgatgtgaaagcccacggctcaaccgtggagggtcattggaaactggggaacttgagtgcagaagaggaaagcggaattccacgtgtagcggtgaaatgcgtagagatgtggaggaacaccagtggcgaaggcggctttctggtctgtaactgacgctgaggcgcgaaagcgtggggagcaaacaggattagataccctggtagtccacgccgtaaacgatgagtgctaagtgttagagggtttccgccctttagtgctgcagctaacgcattaagcactccgcctggggagtacggccgcaaggctgaaactcaaaggaattgacgggggcccgcacaagcggtggagcatgtggtttaattcgaagcaacgcgaagaaccttaccaggtcttgacatcctttgaccactctagagatagagctttccccttcgggggacaaagtgacaggtggtgcatggttgtcgtcagctcgtgtcgtgagatgttgggttaagtcccgcaacgagcgcaacccttgatcttagttgccagcattaagttgggcactctaaggtgactgccggtgacaaaccggaggaaggtggggatgacgtcaaatcatcatgccccttatgacctgggctacacacgtgctacaatggatgatacaaagggttgcgaagccgcgaggtgaagctaatctcataaaatcattctcagttcggattgtaggctgcaactcgcctacatgaagctggaatcgctagtaatcgcggatcagcatgccgcggtgaatacgttcccgggccttgtacacaccgcccgtcacaccacgagagtttgtaacacccgaagtcggtggggtaaccgtaaggagccagccgcctaaggtgggacagatgattggggtgaagtcgtaacaaggtagccgtatcggaaggtgcggctggatcacctccttt

SEQ ID NO: 11 - DNA, 1454 bp, Bacillus drentensis
  source 1..1454: mol_type = unassigned DNA
cttggagagtttgatcctggctcaggacgaacgctggcggcgtgcctaatacatgcaagtcgagcgaatcttcaggagcttgctcctgttggttagcggcggacgggtgagtaacacgtgggcaacctgcctgtaagactgggataacaccgggaaaccggtgctaataccggataatccttttcctctcatgaggaaaagctgaaagtcggtttcggctgacacttacagatgggcccgcggcgcattagctagttggtgaggtaacggctcaccaaggcgacgatgcgtagccgacctgagagggtgatcggccacactgggactgagacacggcccagactcctacgggaggcagcagtagggaatcttccacaatggacgaaagtctgatggagcaacgccgcgtgagcgatgaaggccttcgggtcgtaaagctctgttgttagggaagaacaagtaccggagtaactgccggtaccttgacggtacctaaccagaaagccacggctaactacgtgccagcagccgcggtaatacgtaggtggcaagcgttgtccggaattattgggcgtaaagcgcgcgcaggcggtcctttaagtctgatgtgaaagcccacggctcaaccgtggagggtcattggaaactgggggacttgagtgcagaagaggaaagcggaattccacgtgtagcggtgaaatgcgtagagatgtggaggaacaccagtggcgaaggcggctttctggtctgtaactgacgctgaggcgcgaaagcgtggggagcaaacaggattagataccctggtagtccacgccgtaaacgatgagtgctaagtgttagggggtttccgccccttagtgctgcagctaacgcattaagcactccgcctggggagtacggccgcaaggctgaaactcaaaggaattgacgggggcccgcacaagcggtggagcatgtggtttaattcgaagcaacgcgaagaaccttaccaggtcttgacatcctctgacactcctagagataggacgttccccttcgggggacagagtgacaggtggtgcatggttgtcgtcagctcgtgtcgtgagatgttgggttaagtcccgcaacgagcgcaacccttgatcttagttgccagcattcagttgggcactctaaggtgactgccggtgacaaaccggaggaaggtggggatgacgtcaaatcatcatgccccttatgacctgggctacacacgtgctacaatggatggtacaaagggctgcaagaccgcgaggtttagccaatcccataaaaccattctcagttcggattgcaggctgcaactcgcctgcatgaagccggaatcgctagtaatcgcggatcagcatgccgcggtgaatacgttcccgggccttgtacacaccgcccgtcacaccacgagagtttgtaacacccgaagtcggtggggtaac

SEQ ID NO: 12 - DNA, 1454 bp, Bacillus subtilis; identical to SEQ ID NO: 11
  source 1..1454: mol_type = unassigned DNA

SEQ ID NO: 13 - DNA, 1320 bp, Clostridium bifermentans
  source 1..1320: mol_type = unassigned DNA
gcttttgtatcaaagctccggcggtacaggatggacccgcgtctgattagctagttggtaaggtaatggcttaccaaggcaacgatcagtagccgacctgagagggtgatcggccacactggaactgagacacggtccagactcctacgggaggcagcagtggggaatattgcacaatgggcgaaagcctgatgcagcaacgccgcgtgagcgatgaaggccttcgggtcgtaaagctctgtcctcaaggaagataatgacggtacttgaggaggaagccccggctaactacgtgccagcagccgcggtaatacgtagggggctagcgttatccggaattactgggcgtaaagggtgcgtaggtggttttttaagtcagaagtgaaaggctacggctcaaccgtagtaagcttttgaaactagagaacttgagtgcaggagaggagagtagaattcctagtgtagcggtgaaatgcgtagatattaggaggaataccagtagcgaaggcggctctctggactgtaactgacactgaggcacgaaagcgtggggagcaaacaggattagataccctggtagtccacgccgtaaacgatgagtactaggtgtcgggggttacccccctcggtgccgcagctaacgcattaagtactccgcctgggaagtacgctcgcaagagtgaaactcaaaggaattgacggggacccgcacaagtagcggagcatgtggtttaattcgaagcaacgcgaagaaccttacctaagcttgacatcccactgacctctccctaatcggagatttcccttcggggacagtggtgacaggtggtgcatggttgtcgtcagctcgtgtcgtgagatgttgggttaagtcccgcaacgagcgcaacccttgcctttagttgccagcattaagttgggcactctagagggactgccgaggataactcggaggaaggtggggatgacgtcaaatcatcatgccccttatgcttagggctacacacgtgctacaatgggtggtacagagggttgccaagccgcgaggtggagctaatcccttaaagccattctcagttcggattgtaggctgaaactcgcctacatgaagctggagttactagtaatcgcagatcagaatgctgcggtgaatgcgttcccgggtcttgtacacaccgcccgtcacaccatggaagttgggggcgcccgaagccggttagctaaccttttaggaagcggccgtcgaaggtgaaaccaatgactggggtgaagtcgtaacaaggtagccgtatcggaaggtgcggctggatcacctccttt

SEQ ID NO: 14 - DNA, 1510 bp, Clostridium beijerinckii
  source 1..1510: mol_type = unassigned DNA
tattgagagtttgatcctggctcaggacgaacgctggcggcgtgcttaacacatgcaagtcgagcgatgaagttccttcgggaatggattagcggcggacgggtgagtaacacgtgggtaacctgcctcatagaggggaatagcctttcgaaaggaagattaataccgcataagattgtagtgccgcatggcatagcaattaaaggagtaatccgctatgagatggacccgcgtcgcattagctagttggtgaggtaacggctcaccaaggcgacgatgcgtagccgacctgagagggtgatcggccacattgggactgagacacggcccagactcctacgggaggcagcagtggggaatattgcacaatgggggaaaccctgatgcagcaacgccgcgtgagtgatgacggtcttcggattgtaaagctctgtcttcagggacgataatgacggtacctgaggaggaagccacggctaactacgtgccagcagccgcggtaatacgtaggtggcaagcgttgtccggatttactgggcgtaaagggagcgtaggtggatatttaagtgggatgtgaaatactcgggcttaacctgggtgctgcattccaaactggatatctagagtgcaggagaggaaagtagaattcctagtgtagcggtgaaatgcgtagagattaggaagaataccagtggcgaaggcgactttctggactgtaactgacactgaggctcgaaagcgtggggagcaaacaggattagataccctggtagtccacgccgtaaacgatgaatactaggtgtaggggttgtcatgacctctgtgccgccgctaacgcattaagtattccgcctggggagtacggtcgcaagattaaaactcaaaggaattgacgggggcccgcacaagcagcggagcatgtggtttaattcgaagcaacgcgaagaaccttacctagacttgacatctcctgaattacccttaatcggggaagcccttcggggcaggaagacaggtggtgcatggttgtcgtcagctcgtgtcgtgagatgttgggttaagtcccgcaacgagcgcaacccttattgttagttgctaccatttagttgagcactctagcgagactgcccgggttaaccgggaggaaggtggggatgacgtcaaatcatcatgccccttatgtctagggctacacacgtgctacaatggctggtacagagagatgctaaaccgtgaggtggagccaaactttaaaaccagtctcagttcggattgtaggctgaaactcgcctacatgaagctggagttgctagtaatcgcgaatcagaatgtcgcggtgaatacgttcccgggccttgtacacaccgcccgtcacaccatgagagttggcaatacccaaagttcgtgagctaacgcgcaagcggggcagcgacctaaggtagggtcagcgattggggtgaagtcgtaacaaggtagccgtaggagaacctgcggctggatcacctccttt

SEQ ID NO: 15 - DNA, 1505 bp, Clostridium pasteurianum
  source 1..1505: mol_type = unassigned DNA
aattgagagtttgatcctggctcaggacgaacgctggcggcgtgcttaacacatgcaagtcgagcgagaaaccttcgggtttctagcggcggacgggtgagtaacacgtgggtaacctgcctcaaagaggggaatagcctcccgaaagggagattaataccgcataatattacagcttcgcatgaagcagtaattaaaggagtaatccgctttgagatggacccgcggcgcattagctagttggagaggtaacggctcaccaaggcgacgatgcgtagccgacctgagagggtgatcggccacattggaactgagacacggtccagactcctacgggaggcagcagtggggaatattgcacaatgggcgaaagcctgatgcagcaacgccgcgtgagtgatgacggtcttcggattgtaaagctctgtcttttgggacgataatgacggtaccaaaggaggaagccacggctaactacgtgccagcagccgcggtaatacgtaggtggcaagcgttgtccggatttactgggcgtaaaggatgtgtaggcggatacttaagtgagatgtgaaagccccgggcttaacttggggactgcatttcaaactgggtgtctagagtgcaggagaggaaagcggaattcctagtgtagcggtgaaatgcgtagagattaggaagaacatcagtggcgaaggcggctttctggactgtaactgacgctgaggcatgaaagcgtggggagcaaacaggattagataccctggtagtccacgccgtaaacgatgagtactaggtgtaggaggtatcgactccttctgtgccgcagtaaacacaataagtactccgcctgggaagtacggtcgcaagattaaaactcaaaggaattgacgggggcccgcacaagcagcggagcatgtggtttaattcgaagcaacgcgaagaaccttacctagacttgacatctcctgaatagcgtagagatacgtgaagcccttcggggcaggaagacaggtggtgcatggttgtcgtcagctcgtgtcgtgagatgttgggttaagtcccgcaacgagcgcaacccttatcattagttgctaccattaagttgagcactctagtgagactgcccgggttaaccgggaggaaggcggggatgacgtcaaatcatcatgccccttatgtctagggctacacacgtgctacaatggtgagaacaacgagatgcaataccgcgaggtggagccaaacttgaaaactcatcccagttcggattgtaggctgaaattcgcctacatgaagttggagttgctagtaatcgcgaatcagaatgtcgcggtgaatacgttcccgggccttgtacacaccgcccgtcacaccatgagagctggtaacacccgaagtccgtgaggtaacctttatggagccagcggccgaaggtgggattagtgattggggtgaagtcgtaacaaggtagccgtaggagaacctgcggctggatcacctccttt

SEQ ID NO: 16 - DNA, 1567 bp, Lactobacillus paracasei
  source 1..1567: mol_type = unassigned DNA
tatgagagtttgatcctggctcaggatgaacgctggcggcgtgcctaatacatgcaagtcgaacgagttctcgttgatgatcggtgcttgcaccgagattcaacatggaacgagtggcggacgggtgagtaacacgtgggtaacctgcccttaagtgggggataacatttggaaacagatgctaataccgcatagatccaagaaccgcatggttcttggctgaaagatggcgtaagctatcgcttttggatggacccgcggcgtattagctagttggtgaggtaacggctcaccaaggcgatgatacgtagccgaactgagaggttgatcggccacattgggactgagacacggcccaaactcctacgggaggcagcagtagggaatcttccacaatggacgcaagtctgatggagcaacgccgcgtgagtgaagaaggctttcgggtcgtaaaactctgttgttggagaagaatggtcggcagagtaactgttgtcggcgtgacggtatccaaccagaaagccacggctaactacgtgccagcagccgcggtaatacgtaggtggcaagcgttatccggatttattgggcgtaaagcgagcgcaggcggttttttaagtctgatgtgaaagccctcggcttaaccgaggaagcgcatcggaaactgggaaacttgagtgcagaagaggacagtggaactccatgtgtagcggtgaaatgcgtagatatatggaagaacaccagtggcgaaggcggctgtctggtctgtaactgacgctgaggctcgaaagcatgggtagcgaacaggattagataccctggtagtccatgccgtaaacgatgaatgctaggtgttggagggtttccgcccttcagtgccgcagctaacgcattaagcattccgcctggggagtacgaccgcaaggttgaaactcaaaggaattgacgggggcccgcacaagcggtggagcatgtggtttaattcgaagcaacgcgaagaaccttaccaggtcttgacatcttttgatcacctgagagatcaggtttccccttcgggggcaaaatgacaggtggtgcatggttgtcgtcagctcgtgtcgtgagatgttgggttaagtcccgcaacgagcgcaacccttatgactagttgccagcatttagttgggcactctagtaagactgccggtgacaaaccggaggaaggtggggatgacgtcaaatcatcatgccccttatgacctgggctacacacgtgctacaatggatggtacaacgagttgcgagaccgcgaggtcaagctaatctcttaaagccattctcagttcggactgtaggctgcaactcgcctacacgaagtcggaatcgctagtaatcgcggatcagcacgccgcggtgaatacgttcccgggccttgtacacaccgcccgtcacaccatgagagtttgtaacacccgaagccggtggcgtaacccttttagggagcgagccgtctaaggtgggacaaatgattagggtgaagtcgtaacaaggtagccgtaggagaacctgcggctggatcacctccttt

SEQ ID NO: 17 - DNA, 512 bp, Fontibacillus sp. (panacisegetis)
  source 1..512: mol_type = unassigned DNA
ttagcggcggacgggtgagtaacacgtaggtaacctgcctgtaagactgggataactagcggaaacgttagctaataccggataatttattttctcgcatggggaagtaatgaaagacggagcaatctgtcacttgcagatggacctgcggcgcattagctagttggtggggtaacggctcaccaaggcgacgatgcgtagccgacctgagagggtgaacggccacactgggactgagacacggcccagactcctacgggaggcagcagtagggaatcttccgcaatggacgaaagtctgacggagcaacgccgcgtgagtgatgaaggttttcggatcgtaaagctctgttgccagggaagaacgttcggtagagtaactgctaccggagtgacggtacctgagaagaaagccccggctaactacgtgccagcagccgcggtaatacgtagggggcaagcgttgtccggaattattgggcgtaaagcgcgcgcaggcggctatttaagtct

SEQ ID NO: 18 - DNA, 1561 bp, Oceanobacillus oncorhynchi
  source 1..1561: mol_type = unassigned DNA
ttatggagagtttgatcttggctcaggacgaacgctggcggcgtgcctaatacatgcaagtcgagcgcgggaagcgaacggaactcttcggagggaagttcgtggaacgagcggcggacgggtgagtaacacgtaggcaacctgcctgtaagactgggataactcgcggaaacgcgagctaataccggataacactttctatcacctgatggaaagttgaaaggcggcttttgctgtcacttacagatgggcctgcggcgcattagctagttggtgaggtaacggctcaccaaggcgacgatgcgtagccgacctgagagggtgatcggccacactgggactgagacacggcccagactcctacgggaggcagcagtagggaatcttccgcaatggacgaaagtctgacggagcaacgccgcgtgagtgatgaaggttttcggatcgtaaaactctgttgtcagggaagaacaagtacgatagtaactgatcgtaccttgacggtacctgaccagaaagccacggctaactacgtgccagcagccgcggtaatacgtaggtggcaagcgttgtccggaattattgggcgtaaagcgctcgcaggcggttctttaagtctgatgtgaaatcttgcggctcaaccgcaaacgtgcattggaaactggaggacttgagtgcagaagaggagagtggaattccacgtgtagcggtgaaatgcgtagagatgtggaggaacaccagtggcgaaggcgactctctggtctgtaactgacgctgaggagcgaaagcgtggggagcgaacaggattagataccctggtagtccacgccgtaaacgatgagtgctaggtgttagggggtttccgccccttagtgctgaagttaacgcattaagcactccgcctggggagtacggccgcaaggctgaaactcaaaagaattgacggggacccgcacaagcggtggagcatgtggtttaattcgaagcaacgcgaagaaccttaccaggtcttgacatcctttgaccgctctagagatagagttttcccttcggggacaaagtgacaggtggtgcatggttgtcgtcagctcgtgtcgtgagatgttgggttaagtcccgcaacgagcgcaacccttaatcttagttgccagcatttagttgggcactctaaggtgactgccggtgacaaaccggaggaaggtggggatgacgtcaaatcatcatgccccttatgacctgggctacacacgtgctacaatggacggaacaaagggaagcgaacccgcgaggtccagcaaatcccataaaaccgttctcagttcggattgcaggctgcaactcgcctgcatgaagccggaatcgctagtaatcgcggatcagcatgccgcggtgaatacgttcccgggtcttgtacacaccgcccgtcacaccacgagagttcgtaacacccgaagtcggtgaggtaaccttttggagccagccgccgaaggtgggacgaatgattggggtgaagtcgtaacaaggtagccgtatcggaaggtgcggctggatcacctccttt

SEQ ID NO: 19 - DNA, 1553 bp, Paenibacillus lautus
  source 1..1553: mol_type = unassigned DNA
attggagagtttgatcctggctcaggacgaacgctggcggcgtgcctaatacatgcaagtcgagcggacttgatggagtgcttgcactcctgaaggttagcggcggacgggtgagtaacacgtaggcaacctgccctcaagactgggataactaccggaaacggtagctaataccggataatttattttgcagcattgtgaaataatgaaaggcggagcaatctgtcacttgaggatgggcctgcggcgcattagctagttggtggggtaacggcccaccaaggcgacgatgcgtagccgacctgagagggtgaacggccacactgggactgagacacggcccagactcctacgggaggcagcagtagggaatcttccgcaatgggcgaaagcctgacggagcaacgccgcgtgagtgatgaaggttttcggatcgtaaagctctgttgccaaggaagaacgtcttctagagtaactgctaggagagtgacggtacttgagaagaaagccccggctaactacgtgccagcagccgcggtaatacgtagggggcaagcgttgtccggaattattgggcgtaaagcgcgcgcaggcggttctttaagtctggtgtttaaacccgaggctcaacttcgggtcgcactggaaactggggaacttgagtgcagaagaggagagtggaattccacgtgtagcggtgaaatgcgtagatatgtggaggaacaccagtggcgaaggcgactctctgggctgtaactgacgctgaggcgcgaaagcgtggggagcaaacaggattagataccctggtagtccacgccgtaaacgatgaatgctaggtgttaggggtttcgatacccttggtgccgaagttaacacattaagcattccgcctggggagtacggtcgcaagactgaaactcaaaggaattgacggggacccgcacaagcagtggagtatgtggtttaattcgaagcaacgcgaagaaccttaccaagtcttgacatccctctgaatcctctagagatagaggcggccttcgggacagaggtgacaggtggtgcatggttgtcgtcagctcgtgtcgtgagatgttgggttaagtcccgcaacgagcgcaacccttgattttagttgccagcacttcgggtgggcactctagaatgactgccggtgacaaaccggaggaaggcggggatgacgtcaaatcatcatgccccttatgacttgggctacacacgtactacaatggctggtacaacgggaagcgaagccgcgaggtggagccaatcctataaaagccagtctcagttcggattgcaggctgcaactcgcctgcatgaagtcggaattgctagtaatcgcggatcagcatgccgcggtgaatacgttcccgggtcttgtacacaccgcccgtcacaccacgagagtttacaacacccgaagtcggtggggtaacccttaggggagccagccgccgaaggtggggtagatgattggggtgaagtcgtaacaaggtagccgtatcggaaggtgcggctggatcacctccttt

SEQ ID NO: 20 - DNA, 1553 bp, Paenibacillus chibensis
  source 1..1553: mol_type = unassigned DNA
cttggagagtttgatcctggctcaggacgaacgctggcggcgtgcctaatacatgcaagtcgagcggagttgatgaggtgcttgcacctctgatgcttagcggcggacgggtgagtaacacgtaggtaacctgcctgtaagactgggataactaccggaaacggtagctaataccggataatttattttctctcctggggagataatgaaagacggagcaatctgtcacttacagatgggcctgcggcgcattagctagttggtgaggtaacggctcaccaaggcgacgatgcgtagccgacctgagagggtgaacggccacactgggactgagacacggcccagactcctacgggaggcagcagtagggaatcttccgcaatggacgaaagtctgacggagcaacgccgcgtgagtgatgaaggttttcggatcgtaaagctctgttgccagggaagaacgtccggtagagtaactgctaccggagtgacggtacctgagaagaaagccccggctaactacgtgccagcagccgcggtaatacgtagggggcaagcgttgtccggaattattgggcgtaaagcgcgcgcaggcggtcacttaagtctggtgtttaaggccaaggctcaaccttggttcgcactggaaactgggtgacttgagtgcagaagaggagagtggaattccacgtgtagcggtgaaatgcgtagatatgtggaggaacaccagtggcgaaggcgactctctgggctgtaactgacgctgaggcgcgaaagcgtggggagcaaacaggattagataccctggtagtccacgccgtaaacgatgaatgctaggtgttaggggtttcgatacccttggtgccgaagttaacacattaagcattccgcctggggagtacggtcgcaagactgaaactcaaaggaattgacggggacccgcacaagcagtggagtatgtggtttaattcgaagcaacgcgaagaaccttaccaagtcttgacatccctctgaatcctctagagatagaggcggccttcgggacagaggtgacaggtggtgcatggttgtcgtcagctcgtgtcgtgagatgttgggttaagtcccgcaacgagcgcaacccttgattttagttgccagcatttcggatgggcactctagaatgactgccggtgacaaaccggaggaaggcggggatgacgtcaaatcatcatgccccttatgacttgggctacacacgtactacaatggccagtacaacgggaagcgaaatcgcgagatggagccaatcctatcaaagctggtctcagttcggattgcaggctgcaacccgcctgcatgaagtcggaattgctagtaatcgcggatcagcatgccgcggtgaatacgttcccgggtcttgtacacaccgcccgtcacaccacgagagtttacaacacccgaagtcggtggggtaacccgcaagggagccagccgccgaaggtggggtagatgattggggtgaagtcgtaacaaggtagccgtatcggaaggtgcggctggatcacctccttt

SEQ ID NO: 21 - DNA, 1552 bp, Paenibacillus cookii
  source 1..1552: mol_type = unassigned DNA
cttggagagtttgatcctggctcaggacgaacgctggcggcgtgcctaatacatgcaagtcgagcggagttgatggggagcttgctctcctgagacttagcggcggacgggtgagtaacacgtaggcaacctgcccgtaagaccgggataactaccggaaacggtagctaataccggataatttatcgcttcgcatggagcggtaatgaaagacggagcaatctgtcacttacggatgggcctgcggcgcattagctagttggtgaggtaacggctcaccaaggcgacgatgcgtagccgacctgagagggtgaacggccacactgggactgagacacggcccagactcctacgggaggcagcagtagggaatcttccgcaatgggcgaaagcctgacggagcaacgccgcgtgagtgatgaaggttttcggatcgtaaagctctgttgccagggaagaacgtcgggtagagtaactgctatccgagtgacggtacctgagaagaaagccccggctaactacgtgccagcagccgcggtaatacgtagggggcaagcgttgtccggaattattgggcgtaaagcgcgcgcaggcggtcacttaagtctggtgtttaaggctagggctcaactctagttcgcactggaaactgggtgacttgagtgcagaagaggaaagtggaattccacgtgtagcggtgaaatgcgtagagatgtggaggaacaccagtggcgaaggcgactttctgggctgtaactgacgctgaggcgcgaaagcgtggggagcaaacaggattagataccctggtagtccacgccgtaaacgatgaatgctaggtgttaggggtttcgatacccttggtgccgaagttaacacattaagcattccgcctggggagtacggtcgcaagactgaaactcaaaggaattgacggggacccgcacaagcagtggagtatgtggtttaattcgaagcaacgcgaagaaccttaccaggtcttgacatccctctgaatcctctagagatagaggcggccttcgggacagaggagacaggtggtgcatggttgtcgtcagctcgtgtcgtgagatgttgggttaagtcccgcaacgagcgcaacccttgattttagttgccagcacattaaggtgggcactctagaatgactgccggtgacaaaccggaggaaggcggggatgacgtcaaatcatcatgccccttatgacctgggctacacacgtactacaatggccagtacaacgggaagcgaagtcgcgagacggagccaatcctatcaaagctggtctcagttcggattgcaggctgcaacccgcctgcatgaagtcggaattgctagtaatcgcggatcagcatgccgcggtgaatacgttcccgggtcttgtacacaccgcccgtcacaccacgagagtttacaacacccgaagtcggtggggtaaccgcaaggagccagccgccgaaggtggggtagatgattggggtgaagtcgtaacaaggtagccgtatcggaaggtgcggctggatcacctccttt

SEQ ID NO: 22 - DNA, 1330 bp, Paenibacillus sp. (chitinolyticus)
  source 1..1330: mol_type = unassigned DNA
ctgtggcttacggatgggcctgcggcgcattagctagttggtgaggtaacggctcaccaaggcgacgatgcgtagccgacctgagagggtgaacggccacactgggactgagacacggcccagactcctacgggaggcagcagtagggaatcttccgcaatggacgcaagtctgacggagcaacgccgcgtgagtgatgaaggttttcggatcgtaaagctctgttgccagggaagaacgccaaggagagtaactgctctttgggtgacggtacctgagaagaaagccccggctaactacgtgccagcagccgcggtaatacgtagggggcaagcgttgtccggaattattgggcgtaaagcgcgcgcaggcggttttttaagtctggtgtttaatcccgaggctcaacctcggttcgcaccggaaactgggagactggagtgcaggagaggaaagtggaattccacgtgtagcggtgaaatgcgtagagatgtggaggaacaccagtggcgaaggcgactttctggcctgtaactgacgctgaggcgcgaaagcgtggggagcaaacaggattagataccctggtagtccacgccgtaaacgatgaatgctaggtgttaggggtttcgatacccttggtgccgaagttaacacagtaagcattccgcctggggagtacgctcgcaagagtgaaactcaaaggaattgacggggacccgcacaagcagtggagtatgtggtttaattcgaagcaacgcgaagaaccttaccaggtcttgacatccctctgaccggcttagagataagcctttccttcgggacagaggtgacaggtggtgcatggttgtcgtcagctcgtgtcgtgagatgttgggttaagtcccgcaacgagcgcaacccttgaacttagttgccagcaggtaaagctgggcactctaagttgactgccggtgacaaaccggaggaaggcggggatgacgtcaaatcatcatgccccttatgacctgggctacacacgtactacaatggccggtacaacgggaagcgaaggagcgatccggagccaatcctagaaaagccggtctcagttcggattgcaggctgcaactcgcctgcatgaagtcggaattgctagtaatcgcggatcagcatgccgcggtgaatacgttcccgggtcttgtacacaccgcccgtcacaccacgagagtttacaacacccgaagtcggtgaggtaaccgcaaggagccagccgccgaaggtggggtagatgattggggtgaagtcgtaacaaggtagccgtatcggaaggtgcggctggatcacctccttt

SEQ ID NO: 23 - DNA, 866 bp, Paenibacillus sp. (P1PXP2)
  source 1..866: mol_type = unassigned DNA
cagagggatgtcaagacctggtaaggttcttcgcgttgcttcgaattaaaccacatactccactgcttgtgcgggtccccgtcaattcctttgagtttcagtcttgcgaccgtactccccaggcggaatgcttaatgtgttaacttcggcaccaagggtatcgaaacccctaacacctagcattcatcgtttacggcgtggactaccagggtatctaatcctgtttgctccccacgctttcgcgcctcagcgtcagttacagcccagagagtcgccttcgccactggtgttcctccacatatctacgcatttcaccgctacacgtggaattccactctcctcttctgcactcaagtcacccagtttccagtgcgaaccaaggttgagccttggccttaaacaccagacttaaatgaccgcctgcgcgcgctttacgcccaataattccggacaacgcttgccccctacgtattaccgcggctgctggcacgtagttagccggggctttcttctcaggtaccgtcactccgatagcagttactctaccggacgttcttccctggcaacagagctttacgatccgaaaaccttcatcactcacgcggcgttgctccgtcaggctttcgcccattgcggaagattccctactgctgcctcccgtaggagtctgggccgtgtctcagtcccagtgtggccgttcaccctctcaggtcggctacgcatcgtcgccttggtgagccgttacctcaccaactagctaatgcgccgcaggcccatccgcaagtgacagattgctccgtctttcatcatcccctcaggagaggaaatgagatatccggtattagctcacgtttccgtgggttatc

SEQ ID NO: 24 - DNA, 1533 bp, Pseudomonas sp.
  source 1..1533: mol_type = unassigned DNA
ctgaagagtttgatcatggctcagattgaacgctggcggcaggcctaacacatgcaagtcgagcggatgacgggagcttgctccttgattcagcggcggacgggtgagtaatgcctaggaatctgcctggtagtgggggacaacgtttcgaaaggaacgctaataccgcatacgtcctacgggagaaagcaggggaccttcgggccttgcgctatcagatgagcctaggtcggattagctagtaggtgaggtaatggctcacctaggcgacgatccgtaactggtctgagaggatgatcagtcacactggaactgagacacggtccagactcctacgggaggcagcagtggggaatattggacaatgggcgaaagcctgatccagccatgccgcgtgtgtgaagaaggtcttcggattgtaaagcactttaagttgggaggaagggcagtaagctaataccttgctgttttgacgttaccgacagaataagcaccggctaactctgtgccagcagccgcggtaatacagagggtgcaagcgttaatcggaattactgggcgtaaagcgcgcgtaggtggttcgttaagttggatgtgaaagccccgggctcaacctgggaactgcatccaaaactggcgagctagagtatggtagagggtggtggaatttcctgtgtagcggtgaaatgcgtagatataggaaggaacaccagtggcgaaggcgaccacctggactgatactgacactgaggtgcgaaagcgtggggagcaaacaggattagataccctggtagtccacgccgtaaacgatgtcaactagccgttggaatccttgagattttagtggcgcagctaacgcattaagttgaccgcctggggagtacggccgcaaggttaaaactcaaatgaattgacgggggcccgcacaagcggtggagcatgtggtttaattcgaagcaacgcgaagaaccttaccaggccttgacatgcagagaactttccagagatggattggtgccttcgggaactctgacacaggtgctgcatggctgtcgtcagctcgtgtcgtgagatgttgggttaagtcccgtaacgagcgcaacccttgtccttagttaccagcacgttatggtgggcactctaaggagactgccggtgacaaaccggaggaaggtggggatgacgtcaagtcatcatggcccttacggcctgggctacacacgtgctacaatggtcggtacagagggttgccaagccgcgaggtggagctaatctcacaaaaccgatcgtagtccggatcgcagtctgcaactcgactgcgtgaagtcggaatcgctagtaatcgcaaatcagaatgttgcggtgaatacgttcccgggccttgtacacaccgcccgtcacaccatgggagtgggttgcaccagaagtagctagtctaaccttcggggggacggttaccacggtgtgattcatgactggggtgaagtcgtaacaaggtagccgtaggggaacctgcggctggatcacctcctt

SEQ ID NO: 25 - DNA, 1523 bp, Streptomyces griseus
  source 1..1523: mol_type = unassigned DNA
acggagagtttgatcctggctcaggacgaacgctggcggcgtgcttaacacatgcaagtcgaacgatgaagcctttcggggtggattagtggcgaacgggtgagtaacacgtgggcaatctgcccttcactctgggacaagccctggaaacggggtctaataccggataacactctgtcccgcatgggacggggttaaaagctccggcggtgaaggatgagcccgcggcctatcagcttgttggtggggtaatggcctaccaaggcgacgacgggtagccggcctgagagggcgaccggccacactgggactgagacacggcccagactcctacgggaggcagcagtggggaatattgcacaatgggcgaaagcctgatgcagcgacgccgcgtgagggatgacggccttcgggttgtaaacctctttcagcagggaagaagcgagagtgacggtacctgcagaagaagcgccggctaactacgtgccagcagccgcggtaatacgtagggcgcaagcgttgtccggaattattgggcgtaaagagctcgtaggcggcttgtcacgtcggatgtgaaagcccggggcttaaccccgggtctgcattcgatacgggctagctagagtgtggtaggggagatcggaattcctggtgtagcggtgaaatgcgcagatatcaggaggaacaccggtggcgaaggcggatctctgggccattactgacgctgaggagcgaaagcgtggggagcgaacaggattagataccctggtagtccacgccgtaaacgttgggaactaggtgttggcgacattccacgtcgtcggtgccgcagctaacgcattaagttccccgcctggggagtacggccgcaaggctaaaactcaaaggaattgacgggggcccgcacaagcagcggagcatgtggcttaattcgacgcaacgcgaagaaccttaccaaggcttgacatataccggaaagcatcagagatggtgccccccttgtggtcggtatacaggtggtgcatggctgtcgtcagctcgtgtcgtgagatgttgggttaagtcccgcaacgagcgcaacccttgttctgtgttgccagcatgcccttcggggtgatggggactcacaggagactgccggggtcaactcggaggaaggtggggacgacgtcaagtcatcatgccccttatgtcttgggctgcacacgtgctacaatggccggtacaatgagctgcgatgccgcgaggcggagcgaatctcaaaaagccggtctcagttcggattggggtctgcaactcgaccccatgaagtcggagttgctagtaatcgcagatcagcattgctgcggtgaatacgttcccgggccttgtacacaccgcccgtcacgtcacgaaagtcggtaacacccgaagccggtggcccaaccccttgtgggagggagctgtcgaaggtgggactggcgattgggacgaagtcgtaacaaggtagccgtaccggaaggtgcggctggatcacctccttt

SEQ ID NO: 26 - protein, 299 aa, Bacillus megaterium
MLTDLHIAVIGGDARQLEVIRKLIQLDAKTSLIGFDQLDHGFTGATKYQIEELDFSDVDAIILPVPGTNHEGQVDTIFSNEKVVLTEEILKKTPEHCIIYSGISNGYLNELVKTTNRKLVQLFERDDVAIYNSIPTVEGTIMLVIQHTDFTIHGSNISVLGLGRVGMSVARSFAALGANVKVGARKSEHLARIAEMGLQPFYLSELDKEIADSDICINTIPYPILTAKTLSNVPTHALIIDLASKPGGTDFRYAEKRGIKAILAPGLPGIVAPKTAGQIVANVLVNLLKDAADAREEKK

SEQ ID NO: 27 - protein, 297 aa, Bacillus subtilis
MLTGLKIAVIGGDARQLEIIRKLTEQQADIYLVGFDQLDHGFTGAVKCNIDEIPFQQIDSIILPVSATTGEGVVSTVFSNEEVVLKQDHLDRTPAHCVIFSGISNAYLENIAAQAKRKLVKLFERDDIAIYNSIPTVEGTIMLAIQHTDYTIHGSQVAVLGLGRTGMTIARTFAALGANVKVGARSSAHLARITEMGLVPFHTDELKEHVKDIDICINTIPSMILNQTVLSSMTPKTLILDLASRPGGTDFKYAEKQGIKALLAPGLPGIVAPKTAGQILANVLSKLLAEIQAEEGK

SEQ ID NO: 28 - protein, 296 aa, Paenibacillus cookii
MLTGLTIAIIGGDARQLEIIRKLTEQHADIYLAGFDQLDDGFTGTVKCKIDEIPFQKIDSIILPVSATTGEGVVSTVFSNEEVVLKQSYLERTPEHCVIYSGISNAYLEGIASEAGRKLVKLFERDDIAIFNSIPTVEGTIMMAIQHTDYTIHGSNVAVLGMGRTGMTIARTFAALGAKVKVGARSSAHLARITEMGLSPFQLEELTEHVNDIDICINTVPSLILNQSVLSRMTPKTLILDLASRPGGTDFKYAEKQGIKALLAPGLPGIVAPKTAGQIIANVLSKLLADLKKEGK

SEQ ID NO: 29 - protein, 299 aa, Bacillus licheniformis
MLTGLTIAIIGGDARQLEIIRKLTEQDAKVFLIGFDQLDHGFTGATKLKLNELDFGTIDSIILPVSGTSMEGTVATVFSNEKVVLKQEHLEKTKPHCAIYSGISNQYLDGMAKGANRRLIKLFERDDIAIYNSIPTVEGAIMMAIQHTDFTIHGSNVMVLGLGRTGMSISRTFSALGARVKVGARDSAHLARIMEMGLTPFHTNELAEHVENIDICINTIPSLILDKHVLSRMTPRTLILDLATRPGGTDFDFAEKQGIKALLAPGLPGIVAPKTAGQIIANVLCNLLSELTTDRKGLS

SEQ ID NO: 30 - protein, 298 aa, Paenibacillus lautus
MLTGVRTVFVGGDARQIEVIRKCAEMDASVMIAGFEKLQDSFQGVTREPLTPELLSDADALILPVVGCDDEGRVSALFSEGPLRLQEEHIAAMPGHGVIYTGMAKPYLRSLCDKYKIKLVEILERDDVAIYNSIPTAEGALMMAIQNTDFTIHGSTSMVLGMGRTGFTMARSLQGLGAKIRMGVRKSEHYARAEEMGWKPFLVRDLGSYVSDIDLLFNTIPTMIVTAQIISKMPREAVIIDLASAPGGCDFRYAEKRGIKAMLAPGLPGIVAPKTAGIIMANTLVELISEEIKIREDA

SEQ ID NO: 31 - protein, 294 aa, Oceanobacillus oncorhynchi
MSRRIAVIGGDARYLELIKILKSNHDNEVILCGFDKLEQGFTGLNESALDELDQSKLDVVVLPITGTDSKGNVETVFTDKKIHLDEAWFQKLHAECMIFTGMTNAYLTSMAEKAGVTLVPLLDRDDVAIYNSIPTAEGAIMMAFEHTDQTVHSSRVMVVGFGRVGNTVANKFSALGAKVSVCARSIRDLARITEMGLQAVPLHELSNHTENCDILINTIPSLVVTKEAIQNLPTNAVIIDLASKPGGTDFDFAKKRGIQAILARSLPGIVAPRTAGKILANVMEQILEEERASE

SEQ ID NO: 32 - protein, 299 aa, Bacillus amyloliquefaciens
MLTGVQIVFLGGDARQIEVIRKCSEMDATVSVVGFDNLKEKLQGVTRDHLTAELLAAADVLVLPVVGCDDNGIIHTQFSNESLKLQDEHMAALRRGCKVYTGMAKPYLRSLCAHHEIKLIELLDRDEVAISNSIPTSEGALVMAIQNTDFTIHGSNCMVLGLGRTGFTMAKSLQGLGAKVKVGVRSEKDVARAEVMGWEPFLTRDLADHVRNIDLIFNTIPTMIVTAQILSRMPQSAVIIDLASAPGGCDFRYAEKRGIKALLAPGLPGIVAPKTAGSIIANTLVQLISDEFKTRGDGQ

SEQ ID NO: 33 - protein, 300 aa, Bacillus sp.
MLTGLQIAVIGGDARQLEVIRKLTELDAKLYLVGFEQLDHAFSGAVKEKLDEVDFTCIDAIILPVPGAGVDGQIDTIFSNEKITINEEILKKTPQHCKIYSGINPPYLQEISTKADREVVQLFNRDDVAIYNSIPTVEGALMMAIQHTDFTIHGSNVTVLGLGRTGMSIARAFHALGAKVKVGARKSEHIARITEMGLTPFHLSDIEEAVVDTDICINTIPVQVVVASVIAKMPVHTLIIDLASKPGGTDFRYAEKRGVKALLAPGLPGIVAPKTAGRILANVLSQLILANFDEREDKQS

SEQ ID NO: 34 - protein, 299 aa, Paenibacillus chibensis
MLTGVQIVFLGGDARQVEVIRKCSEMDATVSVVGFDNLKQKLQGVTRDHLTAELLAAADVLVLPVVGCDDNGNIHTQFSNEPLKLQDEHMASLRKGCKVYTGMAKPYLRSLCAQHEIKLVELLDRDEVAISNSIPTAEGALVMAIQNTDFTIHGSRCMVLGLGRTGFTMAKSLQGLGAKVKVGVRSEKDVARAEVMGWEPFLTRDLGDHVSNIDLIFNTIPTMIVTAQILSKMPLSSVIIDLASAPGGCDFRYAEKRGIKALLAPGLPGIVAPKTAGLIIAGSLVQLISDEFKTRGDGE

SEQ ID NO: 35 - protein, 299 aa, Bacillus flexus
MLTDLHIAVIGGDARQLEVIRKLIQLDAKTSLIGFDQLDHGFTGATKYQIDELNFSDVDAIILPVPGTNHEGQVDTIFSNEKVILTEEILASTPAHCTIYSGISNDYLNSLVQKTNRTLIQLFERDDVAIYNSIPTVEGTIMLVIQHTDFTIHGANISVLGLGRVGMSVARSFAALGANVKVGARKSEHLARISEMGLTPFHLNDLAQEITDSDICINTIPYPVLTSSVLANIPTHALVVDLASKPGGTDFRYAEKRGIKAILAPGLPGIVAPKTAGQIVANVIVTLLKEAADQREEKQ

SEQ ID NO: 36 - protein, 300 aa, Bacillus firmus
MLTGTQIAVIGGDARQLEIIRKLTELDAKLSLIGFEQLDHAFSGAVKEKIDEVDFSHIDAIILPVPGTGLEGQIETIFSNEKVTLEEEILSQTPAHCTVYSGITNSYLTGVTKSADRRLVQLFERDDVAIYNSIPTVEGTIMMAIQHTDFTIHGSNIAVIGLGRVGMSVARTFRALGAKVKVGARKSEHIARITEMGLTPFNLKEIEDAVKDVDICINTAPHLVVTASVISKMPTHTLIIDLASKPGGTDFRYAEKRGVKALLAPGLPGIVAPKTAGQILANVLSQLIMEDLQKRKGNTK

SEQ ID NO: 37 - protein, 291 aa, Virgibacillus halophilus
MNLKDKKILLIGGDERYLEVVKKLDDLGASVVLAGYDKAGLSSGRVQISKLEDVNFSNLYAILLPVSGTDGEGNITMSSFTDQQLCLTEQMISQLPPSCKIYTGVSGSFLKRMGSKFQKEIISILAREDIAIYNSIPTAEGALQLAMEQTDYTMHSASVMVLGFGKVGMTTARLFSAVGCNVSVAIRKDSAAARVREMGLKPLYTHHLSEEIGQYQIIINTVPDLVLDESLLNIVSSKALIIDLASSPGGVDFSVADELGIRTIHALGLPGKVAPKTAGSIIADTFVSLLS

SEQ ID NO: 38 - protein, 269 aa, Virgibacillus halophilus
MKTIVTGFNKLDQGFTGVQHVEFAEMEHEDIDVVVLPITGTQKGGKVETVFSDEEIVLTKDWFEKFQRPTPVFTGISNQDLDGMVKNSKAQIIPLLDRDDVAIYNSIPTAEGTIMMAMEHTDYTIHSSRVIVAGFGRVGHTVANKFSALGAKVSVAASSIHDIARINEMGLFAITMKELAKAAADCDILINTIPAPVINKEAISQLPHHALIFDLASKPGGTDFDYAKRRGIKAILSESLPGVVAPKTAGKILADVIIQILSQRKGFEQ

SEQ ID NO: 39 - protein, 299 aa, Paenibacillus azoreducens
MLTGVQIVFLGGDARQIEVIRKCSEMDATVSVVGFDNLKEKLQGVTRDQLTGELLAGADVLVLPVVGCDDNGIIHTQFSNESLKLQDEHMASLRRGCKVYTGMAKPYLRSLCAHHEIRLVELLDRDEVAISNSIPTAEGALVMAIQNTDFTIHGSDCMVLGLGRTGFTMAKSLQGLGARVKVGVRSERDFARAEVMGWEPFLTRDLADYVRSIDLIFNTIPTMIVTAQILSRMPQNTVIIDLASAPGGCDFRYAEKRGIKALLAPGLPGIVAPKTAGSIIANSLVQMISDEFKTRGDGE

SEQ ID NO: 40 - protein, 296 aa, synthetic construct
  REGION 1..296: note = Consensus DpaA sequence
TGKHIAVIGGDARQLELIRKLVELGAKVSLVGFDQLDHGFTGATKSSSLEEALSDVDVIILPVPGTNDEGNVDTVFSNEKLVLTEELLELTPEHCTIFSGIANPYLKELAKETNRKLVELFERDDVAILNSIPTAEGAIMMAIEHTPITIHGSNVLVLGFGRTGMTLARTLKALGANVTVGARKSAHLARITEMGLSPFHLSELAEEVGKIDIIFNTIPALVLTKEVLSKMPPEALIIDLASKPGGTDFEYAEKRGIKALLAPGLPGKVAPKTAGQILANVLSQLLAEDLIARKEN

SEQ ID NO: 41 - protein, 296 aa, synthetic construct; identical to SEQ ID NO: 40
  REGION 1..296: note = DpaA consensus sequence

SEQ ID NO: 42 - protein, 201 aa, Bacillus megaterium
MSLKGKRIGFGLTGSHCTYDAVMPEIEKLVNLGAEVLPVVSYTVQSTNTRFGDGEDWVKKIEELTGHAVINTIVKAEPLGPKIPLDCMVVAPITGNTMSKFANAMTESPVLMAAKATLRNNKPVVLGISTNDALGLNGVNLMRLMATKNIYFIPFGQDDPVLKPNSMVARMTMLSDTVYAALEDKQIQPVIVERFRDGQES

SEQ ID NO: 43 - protein, 200 aa, Bacillus subtilis
MSSLKGKRIGFGLTGSHCTYEAVFPQIEALVNEGAEVRPVVTFNVKSTNTRFGEGAEWVKKIEELTGYEAIDSIVKAEPLGPKLPLDCMVIAPLTGNSMSKLANAMTDSPVLMAAKATIRNNRPVVLGISTNDALGLNGTNLMRLMSTKNIFFIPFGQDDPFKKPNSMVAKMDLLPQTIEKALLHQQLQPILVENYQGND

SEQ ID NO: 44 - protein, 196 aa, Paenibacillus cookii
MSLKGKRIGFGLTGSHCTYEEVFPQIEALISQGAEVRPVVTSTVQSTDTRFGEGGDWVRKIEEATGFEAIDSIVKAEPLGPKLPLDCMVIAPLTGNSMSKLANAMTDSPVLMAAKATIRNGRPVVLGISTNDGLGLNGTNLMRLMSAKNIYFIPFGQDDHVKKPTSLVARMDLLPITVEKALLHQQVQPVLVHHHE

SEQ ID NO: 45 - protein, 196 aa, Bacillus licheniformis
MSIKGKRIGFGLTGSHCTYDAVFPQIEALINKGAEVRPVVTHTVKSTDTRFGEGEEWVRRIEELTGFEVIDSIPKAEPLGPKTPLDCMVVAPLTGNSMSKLANAQTDSPVLMAAKATMRNSRPVVLGISTNDALGLNGVNLMRLMAAKNVYFIPFGQDDPYKKPNSLVAKMDLLVPAVEEALSHKQIQPILVHNDQ

SEQ ID NO: 46 - protein, 196 aa, Paenibacillus lautus
MNWNGITVGYALTGSHCTLEEVMPQIQRFKDGGANVVPIVSSTIMTTDTRFGTSENWQKQLKDITGNDIISTIVEAEPLGPSKLLDVLVIAPCTGNTTSKLANAMTDSPVLMAAKAQMRNCRPLVLAISTNDGLGLNAANIAKLLVTKNIYFVPYGQDNPQQKPNSLVAKMNLIPEACYAALEGKQLQPMIVEYSR

SEQ ID NO: 47 - protein, 201 aa, Oceanobacillus oncorhynchi
MTFKNKRIGFGLTGSHHTLPHIFPIIEELIEQGAEVIPFITEMVQYTDTKHGKAADNVKRLEKAANHPIITSIPDAEPYGPDKPLDVMVIAPLTGNSMSKLANAHTDNPVLMAAKSTLRNEHPLLLALTTNDALGLNAKNLAVLLNAKHIYFVPFGQDNPHQKPSSLSANLDQLIPAAEAALKGKQIQPIIVPYSTKNVLK

SEQ ID NO: 48 - protein, 198 aa, Bacillus amyloliquefaciens
MNWQGKTVGYAVTGSHCTLEEIMPQVKRFVEAGANVVPIASGSVQVTDTRFGTAQNWLQQLKDITGNDIITTIVEAEPLGPSKLLDVLVIAPCTGNTTSKLANAMTDSPVLMAAKAQMRNQRPLVLAISTNDGLGLNASNIAKLLITKNIYFVPFGQDNPFQKPNSLVAQMDLIPEACYAALEGKQLQPMILQRVFSA

SEQ ID NO: 49 - protein, 199 aa, Bacillus sp.
MNLKGKKIGFGLTGSHCTYDAVFPEIEKLVGAGAEVIPVVTFTVQNTVTRFGDGEDWIKRIEEVTGNKVIDSIVKAEPLGPKIPLDCMVVAPLTGNSMSKFANAMTDSPVLMAAKATLRNEKPVVLGISTNDALGLNGTNLMRLMSTKNIYFIPFGQDDPVKKPNSMVARMTALSDTIVKAINGEQIQPVIVERYKDGN

SEQ ID NO: 50 - protein, 198 aa, Paenibacillus chibensis
MNWQGKTVGYAITGSHCTLEEIMPQVKRFVDEGAKVVPIVSNSVQVTDTRFGTAQNWLQQLKDITGNDIISSIVDAEPLGPSKLLDVLVIAPCTGNTTSKLANAMTDTPVLMAAKAQMRNLRPLVLAISTNDGLGLNAANIAKLLVTKNIYFVPFGQDNPLQKPNSLVAQMDLIPEACYAALEGRQLQPMILQRIFSA

SEQ ID NO: 51 - protein, 197 aa, Bacillus flexus
MSLKGKRIGFGLTGSHCTYDAVMPEIEKLVNLGAEVMPVVSYTVQSTNTRFGDGEDWIRKIEEVTGNSVINTIVKAEPLGPKIPLDCMVVAPITGNTMSKFANAMTESPVLMAAKATLRNNKPVVLGISTNDALGLNGVNLMRLMATKNIYFIPFGQDDPVSKPNSMVARMPMLSDTVYAALEGKQIQPVVVERFRD

SEQ ID NO: 52 - protein, 199 aa, Bacillus firmus
MSLKGKRIGFGLTGSHCTYDAVFPEIERLVLAGAEVLPVVTFTVKSTETRFGKGEDWVQRIEDLTGNKVIDSIVKAEPLGPKIPLDCMVIAPLTGNTMSKFANAMTDSPVLMAAKATLRNGKPVVLGISTNDALGLNGVNLMRLMATKNIYFIPYGQDDPVKKPNSMVARMTALYDTVIHAMEGKQLQPVLVERYKDES

SEQ ID NO: 53 - protein, 196 aa, Virgibacillus halophilus
MSLDGKRIGFGLTASHCTYEAVFPEMERLINMGAEVVPVVTYNVKNVDTKFGKASDHIKRLEEITNKEVVATIPDAEPLGPITPLDCMVIAPLTGNSMSRLANAITDSPPLMAAKATMRNQNPVVLGISTNDALGLNGVNLMKLMASKMIYFIPFGQDDPVKKPNSLVSDMTLLPETIESALNGNQLQPVLIPFQS

SEQ ID NO: 54 - protein, 198 aa, Paenibacillus azoreducens
MNWQGKTVGYAITGSHCTLEEIMPQVKRFVDEGAKVVPIVSNTVQVTDTRFGTAHNWLQRLKDITGSELISTIVEAEPLGPSKLLDVLVIAPCTGNTTSKLANAITDSPVLMAAKAQMRNLRPLVLAISTNDGLGLNAANIAKLLVAKNIYFVPFGQDNPHQKPNSLVAQMDLIPEACYAALEGRQLQPMLLQRIFSA

SEQ ID NO: 55 - protein, 202 aa, synthetic construct
  REGION 1..202: note = DpaB consensus sequence
  REGION 3..4: note = MISC_FEATURE - X is any amino acid
  REGION 21..22: note = MISC_FEATURE - X is any amino acid
  SITE 24: note = MISC_FEATURE - X is any amino acid
  SITE 26: note = MISC_FEATURE - X is any amino acid
  SITE 29: note = MISC_FEATURE - X is any amino acid
  REGION 32..33: note = MISC_FEATURE - X is any amino acid
  SITE 38: note = MISC_FEATURE - X is any amino acid
  SITE 40: note = MISC_FEATURE - X is any amino acid
  REGION 42..43: note = MISC_FEATURE - X is any amino acid
  SITE 47: note = MISC_FEATURE - X is any amino acid
  REGION 54..57: note = MISC_FEATURE - X is any amino acid
  REGION 59..62: note = MISC_FEATURE - X is any amino acid
  REGION 64..65: note = MISC_FEATURE - X is any amino acid
  REGION 68..70: note = MISC_FEATURE - X is any amino acid
  REGION 72..73: note = MISC_FEATURE - X is any amino acid
  SITE 76: note = MISC_FEATURE - X is any amino acid
  REGION 83..84: note = MISC_FEATURE - X is any amino acid
  SITE 94: note = MISC_FEATURE - X is any amino acid
  SITE 98: note = MISC_FEATURE - X is any amino acid
  SITE 119: note = MISC_FEATURE - X is any amino acid
  REGION 122..123: note = MISC_FEATURE - X is any amino acid
  SITE 128: note = MISC_FEATURE - X is any amino acid
  REGION 139..140: note = MISC_FEATURE - X is any amino acid
  REGION 143..144: note = MISC_FEATURE - X is any amino acid
  REGION 146..147: note = misc_feature - Xaa can be any naturally occurring amino acid
  SITE 154: note = MISC_FEATURE - X is any amino acid
  REGION 162..163: note = MISC_FEATURE - X is any amino acid
  SITE 171: note = MISC_FEATURE - X is any amino acid
  SITE 173: note = MISC_FEATURE - X is any amino acid
  REGION 176..181: note = MISC_FEATURE - X is any amino acid
  SITE 184: note = MISC_FEATURE - X is any amino acid
  SITE 186: note = MISC_FEATURE - X is any amino acid
  SITE 188: note = MISC_FEATURE - X is any amino acid
  REGION 191..192: note = MISC_FEATURE - X is any amino acid
  REGION 194..202: note = MISC_FEATURE - X is any amino acid
MMXXKGKRIGFGLTGSHCTYXXVXPXIEXLVXXGAEVXPXVXXTVQXTDTRFGXXXXWXXXXEXXTGXXXIXXIVXAEPLGPXXPLDCMVIAPXTGNXMSKLANAMTDSPVLMAAKATXRNXXPVVLXISTNDALGLNXXNLXXLXXTKNIYFXPFGQDDPXXKPNSLVAXMXLLXXXXXXALXGXQXQPXXVXXXXXXXXX

SEQ ID NO: 56 - protein, 196 aa, synthetic construct
  REGION 1..196: note = DpaB consensus sequence
MSLKGKRIGFGLTGSHCTYDEVMPEIEKLVDEGAEVTPIVSYTVQTTDTRFGKAEEWIKKIEEITGNKVINTIVEAEPLGPKKLLDCMVIAPCTGNTMAKLANAITDSPVLMAAKATLRNQRPVVLAISTNDALGLNAKNLGRLLNTKNIYFVPFGQDDPVKKPNSLVARMDLLIDTVEEALEGKQLQPVLIEYFR

SEQ ID NO: 57 - protein, 218 aa, Clostridium beijerinckii
MKIYGINGSPRKNKNTATLLQKALDGVKEAAKDKEIETEIINLYDLNYTGCISCFACKRLGSNSYGKCAVKDDLQEVLEKVSQSDGLIFSSPVYFSNVTGKFLSFLERLLFPYLVYDNNGTSLAPKRMPTAFIYTMNVKEEVMKQIGYLKTFERMESNIGHIFTKPLVMYSNNTYQFDDYSKYKVESFSEEEKAAHRKIQFPLDCQKAFELGANLIKH

SEQ ID NO: 58 - protein, 193 aa, Clostridium beijerinckii
MSKVVIFNGSPRKNGYTTKLLEQVAKGAKSKGAEIIEFDLNDSGIRGCQGCFYCRTHDGCAVKDYLQPMYKAITEADAIVFGSPIYYYQITGQAKIWLDRTFPMVGDNFAPRHSGKKLITIFTQGSQNPEMGAEGIKFVNNMLAAYGWKLEDSILCCGTTNFHSEKLGRYDSNLEQFEELSLRAFKDGENLVR

SEQ ID NO: 59 - protein, 183 aa, Clostridium beijerinckii
MSKVVIFKGSPRKNGYTARLLEQVAKGAKSKGAEVIEFDLNDSGIRGCQGCMYCRTHDGCAVNDYLQPMYAAIKEADAIVFGSPIYYYTITGQSKVWFDRTFPMIGNDYKAKYPGKKLITIFTQGNPDPKIGAEGVKFANNMLEELGWKLEDSIHYCGTSHNPDLAMFDELSLRAFKDGENLA

SEQ ID NO: 60 - protein, 182 aa, Clostridium beijerinckii
MSKVVIFKGSPRKNGYTTKLLDQVAKGAKSKGAEVIEFDLNDTGIRGCQGCFYCRTHDGCAVNDYLQPMYKAIAEADAIVFGSPIYMFQITSQAKTCLDRTFPMVEELPNKFIPRHPGKKLITVFAQGSLDPKKGAEAIKYVNNIFDVFGWKLEDCIHYCGTDDEVFNELSLRAFKDGENLA

SEQ ID NO: 61 - protein, 193 aa, Clostridium beijerinckii
MNIIGISASSRKEGNTAWIVNKILEGAKEQGAETQYFDFNNLDIKPCQGCWACHKGDQGCVIKDDMQKLNDAIDRANVIVFGSPIYMMQMSAQGKIIIDRMFARFSPRYSPYFKEESAAEKRLVLTFNQGNPDPELFKSYIDYTKHMFELLEFDVTEVPVVTGLRNGPANEREDLNIMLKDVGKTIVSEGISK

SEQ ID NO: 62 - protein, 208 aa, Clostridium beijerinckii
MKVLLINGSPKAKGCTYTTLCEVADELEKENIETEIFQIGNKPISGCIDCGGCYKSGEGKCVFSDDIVNIALEKAKEADGFIFGSPVHYAAPSGSITSFLDRFFYAGNCFAHKPGAAVVSCRRGGAASAFDQLNKYFTISNMPVVSSQYWNMVHGNTPEEVKQDLEGMQTMRMLGKNMAWLLKSIDAGKKAGISLPESEPRVATNFIR

SEQ ID NO: 63 - protein, 201 aa, Archaeoglobus fulgidus
MKLLAINGSPNKRNTLFLLEVIAEEVKKLGHEAEIIHLKDYEIKECKGCDACLKGDCSQKDDIYKVLEKMQEADAIVIGTPTYFGNVTGIVKNLIDRSRMARMGNYRLRNRVFAPVVTSGLRNGGAEYAAMSLIVYALGQAMLPVSIVENPITTGTFPVGVIQGDAGWRSVKKDEIAINSAKALAKRIVEVAEATKNLRES

SEQ ID NO: 64 - protein, 193 aa, Methanocaldococcus jannaschii
MKVIGISGSPRPEGNTTLLVREALNAIAEEGIETEFISLADKELNPCIGCNMCKEEGKCPIIDDVDEILKKMKEADGIILGSPVYFGGVSAQLKMLMDRSRPLRIGFQLRNKVGGAVAVGASRNGGQETTIQQIHNFFLIHSMIVVGDNDPTAHYGGTGVGKAPGDCKNDDIGLETARNLGKKVAEVVKLIKK

SEQ ID NO: 65 - protein, 225 aa, Peptoclostridium difficile
MIITVINGSPRKNGATSKVLTYLYKDIERLIPDVKINYFDLSEVNPSYCIGCLNCYKMGKCINQNDKVEYIHDIITKSDGVIFGSPTYGSSVTGLFKVFTDRAHMMLERLLYRKPCIAVTTYENARGSKAISFIKSMVLDSGGYVCGSLSIKTGFNQNPITEKVESKIQKVSKKFIYCIEEKKNPPVLSQIYNFIAINAVLKPMAFKDIEQYKGIIDRWEEQGII

SEQ ID NO: 66 - protein, 191 aa, Methanosarcina thermophila
MKITGISGSPRKGQNCEKIIGAALEVAKERGFETDTVFISNEEVAPCKACGACRDQDFCVIDDDMDEIYEKMRAADGIIVAAPVYMGNYPAQLKALFDRSVLLRRKNFALKNKVGAALSVGGSRNGGQEKTIQSIHDWMHIHGMIVVGDNSHFGGITWNPAEEDTVGMQTVSETAKKLCDVLELIQKNRDK

SEQ ID NO: 67 - protein, 289 aa, synthetic construct
  REGION 1..289: note = Consensus Isf sequence
  REGION 4..6: note = MISC_FEATURE - X is any amino acid
  SITE 8: note = MISC_FEATURE - X is any amino acid
  SITE 14: note = MISC_FEATURE - X is any amino acid
  SITE 16: note = MISC_FEATURE - X is any amino acid
  REGION 18..19: note = MISC_FEATURE - X is any amino acid
  REGION 22..28: note = MISC_FEATURE - X is any amino acid
  SITE 34: note = MISC_FEATURE - X is any amino acid
  SITE 37: note = MISC_FEATURE - X is any amino acid
  SITE 39: note = MISC_FEATURE - X is any amino acid
  REGION 41..43: note = MISC_FEATURE - X is any amino acid
  SITE 45: note = MISC_FEATURE - X is any amino acid
  SITE 47: note = MISC_FEATURE - X is any amino acid
  REGION 49..50: note = MISC_FEATURE - X is any amino acid
  REGION 52..53: note = MISC_FEATURE - X is any amino acid
  SITE 55: note = MISC_FEATURE - X is any amino acid
  REGION 58..59: note = MISC_FEATURE - X is any amino acid
  REGION 61..64: note = MISC_FEATURE - X is any amino acid
  REGION 68..70: note = MISC_FEATURE - X is any amino acid
  REGION 72..74: note = MISC_FEATURE - X is any amino acid
  REGION 77..79: note = MISC_FEATURE - X is any amino acid
  REGION 81..86: note = MISC_FEATURE - X is any amino acid
  SITE 90: note = MISC_FEATURE - X is any amino acid
  SITE 92: note = MISC_FEATURE - X is any amino acid
  SITE 97: note = MISC_FEATURE - X is any amino acid
  REGION 99..102: note = MISC_FEATURE - X is any amino acid
  SITE 106: note = MISC_FEATURE - X is any amino acid
  REGION 108..110: note = MISC_FEATURE - X is any amino acid
  REGION 113..136: note = MISC_FEATURE - X is any amino acid
  SITE 140: note = MISC_FEATURE - X is any amino acid
  REGION 152..154: note = MISC_FEATURE - X is any amino acid
  REGION 156..166: note = MISC_FEATURE - X is any amino acid
  REGION 168..175: note = MISC_FEATURE - X is any amino acid
  REGION 177..181: note = MISC_FEATURE - X is any amino acid
  REGION 183..185: note = MISC_FEATURE - X is any amino acid
  REGION 188..200: note = MISC_FEATURE - X is any amino acid
  REGION 202..205: note = MISC_FEATURE - X is any amino acid
  REGION 207..209: note = MISC_FEATURE - X is any amino acid
  SITE 211: note = MISC_FEATURE - X is any amino acid
  REGION 213..216: note = MISC_FEATURE - X is any amino acid
  REGION 236..241: note = MISC_FEATURE - X is any amino acid
  REGION 243..244: note = MISC_FEATURE - X is any amino acid
  REGION 246..251: note = MISC_FEATURE - X is any amino acid
  REGION 253..255: note = MISC_FEATURE - X is any amino acid
  REGION 257..261: note = MISC_FEATURE - X is any amino acid
  REGION 263..265: note = MISC_FEATURE - X is any amino acid
  REGION 267..272: note = MISC_FEATURE - X is any amino acid
  SITE 276: note = MISC_FEATURE - X is any amino acid
MMKXXXIXGSPRKXGXTXXLLXXXXXXXKEAAKXLIXGXEXXXFXLXDXXIXXCXGCXXCXXXXSNSXXXCXXXDDXXXIXXXXXXEADXIXFGSPXYXXXXTGQXKXXXDRXXXXXXXXXXXXXXXXXXXXXXXXLITXFIYTMNVKEEVXXXGXXXXXXXXXXXNXXXXXXXXMXXXXXNXXXITXXXXXXXXXXXXXGXXXXPXXXKXDXXXXKVSKKFIYCIEEKKNPPVLXXXXXXLXXFXXXXXXAXXXGXXXXXVXXXIXXXXXXGISXPESEPRVATNFIR